European Patent Application EP 4 610 351 A1, published September 3, 2025. Title: Novel variant of pyruvate kinase 2 and method for producing L-aromatic amino acid using the same. Applicant: DAESANG CORPORATION. The sequence listing filed with the application follows.

SEQUENCE LISTING (24 sequences)

SEQ ID NO: 1 - DNA, 1443 bp, Escherichia coli
  source 1..1443: mol_type = genomic DNA
atgtccagaaggcttcgcagaacaaaaatcgttaccacgttaggcccagcaacagatcgcgataataatcttgaaaaagttatcgcggcgggtgccaacgttgtacgtatgaacttttctcacggctcgcctgaagatcacaaaatgcgcgcggataaagttcgtgagattgccgcaaaactggggcgtcatgtggctattctgggtgacctccaggggcccaaaatccgtgtatccacctttaaagaaggcaaagttttcctcaatattggggataaattcctgctcgacgccaacctgggtaaaggtgaaggcgacaaagaaaaagtcggtatcgactacaaaggcctgcctgctgacgtcgtgcctggtgacatcctgctgctggacgatggtcgcgtccagttaaaagtactggaagttcagggcatgaaagtgttcaccgaagtcaccgtcggtggtcccctctccaacaataaaggtatcaacaaacttggcggcggtttgtcggctgaagcgctgaccgaaaaagacaaagcagacattaagactgcggcgttgattggcgtagattacctggctgtctccttcccacgctgtggcgaagatctgaactatgcccgtcgcctggcacgcgatgcaggatgtgatgcgaaaattgttgccaaggttgaacgtgcggaagccgtttgcagccaggatgcaatggatgacatcatcctcgcctctgacgtggtaatggttgcacgtggcgacctcggtgtggaaattggcgacccggaactggtcggcattcagaaagcgttgatccgtcgtgcgcgtcagctaaaccgagcggtaatcacggcgacccagatgatggagtcaatgattactaacccgatgccgacgcgtgcagaagtcatggacgtagcaaacgccgttctggatggtactgacgctgtgatgctgtctgcagaaactgccgctgggcagtatccgtcagaaaccgttgcagccatggcgcgcgtttgcctgggtgcggaaaaaatcccgagcatcaacgtttctaaacaccgtctggacgttcagttcgacaatgtggaagaagctattgccatgtcagcaatgtacgcagctaaccacctgaaaggcgttacggcgatcatcaccatgaccgaatcgggtcgtaccgcgctgatgacctcccgtatcagctctggtctgccaattttcgccatgtcgcgccatgaacgtacgctgaacctgactgctctctatcgtggcgttacgccggtgcactttgatagcgctaatgacggcgtagcagctgccagcgaagcggttaatctgctgcgcgataaaggttacttgatgtctggtgacctggtgattgtcacccagggcgacgtgatgagtaccgtgggttctactaataccacgcgtattttaacggtagagtaa

SEQ ID NO: 2 - protein, 480 aa, Escherichia coli
MSRRLRRTKIVTTLGPATDRDNNLEKVIAAGANVVRMNFSHGSPEDHKMRADKVREIAAKLGRHVAILGDLQGPKIRVSTFKEGKVFLNIGDKFLLDANLGKGEGDKEKVGIDYKGLPADVVPGDILLLDDGRVQLKVLEVQGMKVFTEVTVGGPLSNNKGINKLGGGLSAEALTEKDKADIKTAALIGVDYLAVSFPRCGEDLNYARRLARDAGCDAKIVAKVERAEAVCSQDAMDDIILASDVVMVARGDLGVEIGDPELVGIQKALIRRARQLNRAVITATQMMESMITNPMPTRAEVMDVANAVLDGTDAVMLSAETAAGQYPSETVAAMARVCLGAEKIPSINVSKHRLDVQFDNVEEAIAMSAMYAANHLKGVTAIITMTESGRTALMTSRISSGLPIFAMSRHERTLNLTALYRGVTPVHFDSANDGVAAASEAVNLLRDKGYLMSGDLVIVTQGDVMSTVGSTNTTRILTVE

SEQ ID NO: 3 - DNA, 1443 bp, synthetic construct
  source 1..1443: mol_type = other DNA
atgtccagaaggcttcgcagaacaaaaatcgttaccacgttagacccagcaacagatcgcgataataatcttgaaaaagttatcgcggcgggtgccaacgttgtacgtatgaacttttctcacggctcgcctgaagatcacaaaatgcgcgcggataaagttcgtgagattgccgcaaaactggggcgtcatgtggctattctgggtgacctccaggggcccaaaatccgtgtatccacctttaaagaaggcaaagttttcctcaatattggggataaattcctgctcgacgccaacctgggtaaaggtgaaggcgacaaagaaaaagtcggtatcgactacaaaggcctgcctgctgacgtcgtgcctggtgacatcctgctgctggacgatggtcgcgtccagttaaaagtactggaagttcagggcatgaaagtgttcaccgaagtcaccgtcggtggtcccctctccaacaataaaggtatcaacaaacttggcggcggtttgtcggctgaagcgctgaccgaaaaagacaaagcagacattaagactgcggcgttgattggcgtagattacctggctgtctccttcccacgctgtggcgaagatctgaactatgcccgtcgcctggcacgcgatgcaggatgtgatgcgaaaattgttgccaaggttgaacgtgcggaagccgtttgcagccaggatgcaatggatgacatcatcctcgcctctgacgtggtaatggttgcacgtggcgacctcggtgtggaaattggcgacccggaactggtcggcattcagaaagcgttgatccgtcgtgcgcgtcagctaaaccgagcggtaatcacggcgacccagatgatggagtcaatgattactaacccgatgccgacgcgtgcagaagtcatggacgtagcaaacgccgttctggatggtactgacgctgtgatgctgtctgcagaaactgccgctgggcagtatccgtcagaaaccgttgcagccatggcgcgcgtttgcctgggtgcggaaaaaatcccgagcatcaacgtttctaaacaccgtctggacgttcagttcgacaatgtggaagaagctattgccatgtcagcaatgtacgcagctaaccacctgaaaggcgttacggcgatcatcaccatgaccgaatcgggtcgtaccgcgctgatgacctcccgtatcagctctggtctgccaattttcgccatgtcgcgccatgaacgtacgctgaacctgactgctctctatcgtggcgttacgccggtgcactttgatagcgctaatgacggcgtagcagctgccagcgaagcggttaatctgctgcgcgataaaggttacttgatgtctggtgacctggtgattgtcacccagggcgacgtgatgagtaccgtgggttctactaataccacgcgtattttaacggtagagtaa

SEQ ID NO: 4 - protein, 480 aa, synthetic construct
MSRRLRRTKIVTTLDPATDRDNNLEKVIAAGANVVRMNFSHGSPEDHKMRADKVREIAAKLGRHVAILGDLQGPKIRVSTFKEGKVFLNIGDKFLLDANLGKGEGDKEKVGIDYKGLPADVVPGDILLLDDGRVQLKVLEVQGMKVFTEVTVGGPLSNNKGINKLGGGLSAEALTEKDKADIKTAALIGVDYLAVSFPRCGEDLNYARRLARDAGCDAKIVAKVERAEAVCSQDAMDDIILASDVVMVARGDLGVEIGDPELVGIQKALIRRARQLNRAVITATQMMESMITNPMPTRAEVMDVANAVLDGTDAVMLSAETAAGQYPSETVAAMARVCLGAEKIPSINVSKHRLDVQFDNVEEAIAMSAMYAANHLKGVTAIITMTESGRTALMTSRISSGLPIFAMSRHERTLNLTALYRGVTPVHFDSANDGVAAASEAVNLLRDKGYLMSGDLVIVTQGDVMSTVGSTNTTRILTVE

SEQ ID NO: 5 - DNA, 30 bp, synthetic construct
  source 1..30: mol_type = other DNA
caattttattatagtaattgactattatac

SEQ ID NO: 6 - DNA, 40 bp, synthetic construct
  source 1..40: mol_type = other DNA
agcaacagatcaattttattatagtaattgactattatac

SEQ ID NO: 7 - DNA, 40 bp, synthetic construct
  source 1..40: mol_type = other DNA
atctgttgctgggcctaacggttttagagctagaaatagc

SEQ ID NO: 8 - DNA, 30 bp, synthetic construct
  source 1..30: mol_type = other DNA
gggcctaacggttttagagctagaaatagc

SEQ ID NO: 9 - DNA, 21 bp, synthetic construct
  source 1..21: mol_type = other DNA
gagcctgtcggcctacctgct

SEQ ID NO: 10 - DNA, 20 bp, synthetic construct
  source 1..20: mol_type = other DNA
cggccggcatgagcctgtcg

SEQ ID NO: 11 - DNA, 30 bp, synthetic construct
  source 1..30: mol_type = other DNA
atgccggccgttgtagcgacggagacgtgg

SEQ ID NO: 12 - DNA, 20 bp, synthetic construct
  source 1..20: mol_type = other DNA
ttgtagcgacggagacgtgg

SEQ ID NO: 13 - DNA, 20 bp, synthetic construct
  source 1..20: mol_type = other DNA
taacgatttttgttctgcga

SEQ ID NO: 14 - DNA, 30 bp, synthetic construct
  source 1..30: mol_type = other DNA
taacgatttttgttctgcgaagccttctgg

SEQ ID NO: 15 - DNA, 30 bp, synthetic construct
  source 1..30: mol_type = other DNA
ccacgttagacccagcaacagatcgcgata

SEQ ID NO: 16 - DNA, 20 bp, synthetic construct
  source 1..20: mol_type = other DNA
acccagcaacagatcgcgat

SEQ ID NO: 17 - DNA, 20 bp, synthetic construct
  source 1..20: mol_type = other DNA
aacgccgcagtcttaatgtc

SEQ ID NO: 18 - DNA, 20 bp, synthetic construct
  source 1..20: mol_type = other DNA
tacgccaatcaacgccgcag

SEQ ID NO: 19 - DNA, 33 bp, synthetic construct
  source 1..33: mol_type = other DNA
gattggcgtagagctcctgaaaatctcgataac

SEQ ID NO: 20 - DNA, 23 bp, synthetic construct
  source 1..23: mol_type = other DNA
gagctcctgaaaatctcgataac

SEQ ID NO: 21 - DNA, 20 bp, synthetic construct
  source 1..20: mol_type = other DNA
aatgttccggtggtgtactc

SEQ ID NO: 22 - DNA, 20 bp, synthetic construct
  source 1..20: mol_type = other DNA
ttcgcatcacatcctgcatc

SEQ ID NO: 23 - DNA, 3234 bp, synthetic construct
  source 1..3234: mol_type = other DNA
tttccataggctccgcccccctgacgagcatcacaaaaatcgacgctcaagtcagaggtggcgaaacccgacaggactataaagataccaggcgtttccccctggaagctccctcgtgcgctctcctgttccgaccctgccgcttaccggatacctgtccgcctttctcccttcgggaagcgtggcgctttctcatagctcacgctgtaggtatctcagttcggtgtaggtcgttcgctccaagctgggctgtgtgcacgaaccccccgttcagcccgaccgctgcgccttatccggtaactatcgtcttgagtccaacccggtaagacacgacttatcgccactggcagcagccactggtaacaggattagcagagcgaggtatgtaggcggtgctacagagttcttgaagtggtggcctaactacggctacactagaaggacagtatttggtatctgcgctctgctgaagccagttaccttcggaaaaagagttggtagctcttgatccggcaaacaaaccaccgctggtagcggtggtttttttgtttgcaagcagcagattacgcgcagaaaaaaaggatctcaagaagatcctttgatcttttctacggggtctgacgctcagtggaacgaaaactcacgttaagggattttggtcatgagattatcaaaaaggatcttcacctagatccttttaaattaaaaatgaagttttaaatcaatctaaagtatatatgagtaaacttggtctgacagttaaaagattgacagtataatagtcaattactataataaaattgatgcgcaggtgaaacacctgctgcagttttagagctagaaatagcaagttaaaataaggctagtccgttatcaacttgaaaaagtggcaccgagtcggtgctttttttcgttttccgggacgccctcgcggacgtgctcatagtccacgacgcccgtgattttgtagccctggccgacggccagcaggtaggccgacaggctcatgccggccggagctcctgaaaatctcgataactcaaaaaatacgcccggtagtgatcttatttcattatggtgaaagttggaacctcttaggatcctctagatttaagaaggagatatacataaaactccttctgagctagttctctagcattctattattttgattcgacaccttaataatagcagaaggagtttttacctgtcaaagaaccatcaaacccttgatacacaaggctttgacctaattttgaaaaatgatgttgtttctatatagtatcaagataagaaagaaaaggatttttcgctacgctcaaatcctttcccgtcacgggcttctcagggcgttttatggcgggtctgctatgtggtgctatctgactttttgctgttcagcagttcctgccctctgattttccagtctgaccacttcggattatcccgtgacaggtcattcagactggctaatgcacccagtaaggcagcggtatcatcaacggggtctgacgctcagtggaacgaaaactcacgttaagggattttggtcatgagattatcaaaaaggatcttcacctagatccttttaaattaaaaatgaagttttaaatcaatctaaagtatatatgagtaaacttggtctgacagttaccaatgcttaatcagtgaggcacctatctcagcgatctgtctatttcgttcatccatagttgcctgactccccgtcgtgtagataactacgatacgggagggcttaccatctggccccagtgctgcaatgataccgcgagacccacgctcaccggctccagatttatcagcaataaaccagccagccggaagggccgagcgcagaagtggtcctgcaactttatccgcctccatccagtctattaattgttgccgggaagctagagtaagtagttcgccagttaatagtttgcgcaacgttgttgccattgctacaggcatcgtggtgtcacgctcgtcgtttggtatggcttcattcagctccggttcccaacgatcaaggcgagttacatgatcccccatgttgtgcaaaaaagcggttagctccttcggtcctccgatcgttgtcagaagtaagttggccgcagtgttatcactcatggttatggcagcactgcataattctcttactgtcatgccatccgtaagatgcttttctgtgactggtgagtactcaaccaagtcattctgagaatagtgtatgcggcgaccgagttgctcttgcccggcgtcaatacgggataataccgcgccacatagcagaactttaaaagtgctcatcattggaaaacgttcttcggggcgaaaactctcaaggatcttaccgctgttgagatccagttcgatgtaacccactcgtgcacccaactgatcttcagcatcttttactttcaccagcgtttctgggtgagcaaaaacaggaaggcaaaatgccgcaaaaaagggaataagggcgacacggaaatgttgaatactcatactcttcctttttcaatattattgaagcatttatcagggttattgtctcatgagcggatacatatttgaatgtatttagaaaaataaacaaataggggttccgcgcacatttccccgaaaagtgccaccaaaaaaacacaaaagaccacattttttaatgtggtctttattcttcaactaaagcacccattagttcaacaaacgaaaattggataaagtgggatatttttaaaatatatatttatgttacagtaagctgcctcgcgcgtttcggtgatgacggtgaaaacctctgacacatgcagctcccggagacggtcacagcttgtctgtaagcggatgccgggagcagacaagcccgtcagggcgcgtcagcgggtgttggcgggtgtcggggcgcagccatgacccagtcacgtagcgatagcggagtgtatactggcttaactatgcggcatcagagcagattgtactgagagtgcaccatatgcggtgtgaaataccgcacagatgcgtaaggagaaaataccgcatcaggcgctcttccgcttcctcgctcactgactcgctgcgctcggtcgttcggctgcggcgagcggtatcagctcactcaaaggcggtaatacggttatccacagaatcaggggataacgcaggaaagaacatgtgagcaaaaggccagcaaaaggccaggaaccgtaaaaaggccgcgttgctggcgtt

SEQ ID NO: 24 - DNA, 9656 bp, synthetic construct
  source 1..9656: mol_type = other DNA
aaagccatgacaaaaacgcgtaacaaaagtgtctataatcacggcagaaaagtccacattgattatttgcacggcgtcacactttgctatgccatagcatttttatccataagattagcggatcctacctgacgctttttatcgcaactctctactgtttctccatacccgtttttttgggaattcgagctctaaggaggttataaaaaatggatattaatactgaaactgagatcaagcaaaagcattcactaaccccctttcctgttttcctaatcagcccggcatttcgcgggcgatattttcacagctatttcaggagttcagccatgaacgcttattacattcaggatcgtcttgaggctcagagctgggcgcgtcactaccagcagctcgcccgtgaagagaaagaggcagaactggcagacgacatggaaaaaggcctgccccagcacctgtttgaatcgctatgcatcgatcatttgcaacgccacggggccagcaaaaaatccattacccgtgcgtttgatgacgatgttgagtttcaggagcgcatggcagaacacatccggtacatggttgaaaccattgctcaccaccaggttgatattgattcagaggtataaaacgaatgagtactgcactcgcaacgctggctgggaagctggctgaacgtgtcggcatggattctgtcgacccacaggaactgatcaccactcttcgccagacggcatttaaaggtgatgccagcgatgcgcagttcatcgcattactgatcgttgccaaccagtacggccttaatccgtggacgaaagaaatttacgcctttcctgataagcagaatggcatcgttccggtggtgggcgttgatggctggtcccgcatcatcaatgaaaaccagcagtttgatggcatggactttgagcaggacaatgaatcctgtacatgccggatttaccgcaaggaccgtaatcatccgatctgcgttaccgaatggatggatgaatgccgccgcgaaccattcaaaactcgcgaaggcagagaaatcacggggccgtggcagtcgcatcccaaacggatgttacgtcataaagccatgattcagtgtgcccgtctggccttcggatttgctggtatctatgacaaggatgaagccgagcgcattgtcgaaaatactgcatacactgcagaacgtcagccggaacgcgacatcactccggttaacgatgaaaccatgcaggagattaacactctgctgatcgccctggataaaacatgggatgacgacttattgccgctctgttcccagatatttcgccgcgacattcgtgcatcgtcagaactgacacaggccgaagcagtaaaagctcttggattcctgaaacagaaagccgcagagcagaaggtggcagcatgacaccggacattatcctgcagcgtaccgggatcgatgtgagagctgtcgaacagggggatgatgcgtggcacaaattacggctcggcgtcatcaccgcttcagaagttcacaacgtgatagcaaaaccccgctccggaaagaagtggcctgacatgaaaatgtcctacttccacaccctgcttgctgaggtttgcaccggtgtggctccggaagttaacgctaaagcactggcctggggaaaacagtacgagaacgacgccagaaccctgtttgaattcacttccggcgtgaatgttactgaatccccgatcatctatcgcgacgaaagtatgcgtaccgcctgctctcccgatggtttatgcagtgacggcaacggccttgaactgaaatgcccgtttacctcccgggatttcatgaagttccggctcggtggtttcgaggccataaagtcagcttacatggcccaggtgcagtacagcatgtgggtgacgcgaaaaaatgcctggtactttgccaactatgacccgcgtatgaagcgtgaaggcctgcattatgtcgtgattgagcgggatgaaaagtacatggcgagttttgacgagatcgtgccggagttcatcgaaaaaatggacgaggcactggctgaaattggttttgtatttggggagcaatggcgatgagatctaaagaggagaaaggatctatggataagaaatactcaataggcttagatatcggcacaaatagcgtcggatgggcggtgatcactgatgaatataaggttccgtctaaaaagttcaaggttctgggaaatacagaccgccacagtatcaaaaaaaatcttataggggctcttttatttgacagtggagagacagcggaagcgactcgtctcaaacggacagctcgtagaaggtatacacgtcggaagaatcgtatttgttatctacaggagattttttcaaatgagatggcgaaagtagatgatagtttctttcatcgacttgaagagtcttttttggtggaagaagacaagaagcatgaacgtcatcctatttttggaaatatagtagatgaagttgcttatcatgagaaatatccaactatctatcatctgcgaaaaaaattggtagattctactgataaagcggatttgcgcttaatctatttggccttagcgcatatgattaagtttcgtggtcattttttgattgagggagatttaaatcctgataatagtgatgtggacaaactatttatccagttggtacaaacctacaatcaattatttgaagaaaaccctattaacgcaagtggagtagatgctaaagcgattctttctgcacgattgagtaaatcaagacgattagaaaatctcattgctcagctccccggtgagaagaaaaatggcttatttgggaatctcattgctttgtcattgggtttgacccctaattttaaatcaaattttgatttggcagaagatgctaaattacagctttcaaaagatacttacgatgatgatttagataatttattggcgcaaattggagatcaatatgctgatttgtttttggcagctaagaatttatcagatgctattttactttcagatatcctaagagtaaatactgaaataactaaggctcccctatcagcttcaatgattaaacgctacgatgaacatcatcaagacttgactcttttaaaagctttagttcgacaacaacttccagaaaagtataaagaaatcttttttgatcaatcaaaaaacggatatgcaggttatattgatgggggagctagccaagaagaattttataaatttatcaaaccaattttagaaaaaatggatggtactgaggaattattggtgaaactaaatcgtgaagatttgctgcgcaagcaacggacctttgacaacggctctattccccatcaaattcacttgggtgagctgcatgctattttgagaagacaagaagacttttatccatttttaaaagacaatcgtgagaagattgaaaaaatcttgacttttcgaattccttattatgttggtccattggcgcgtggcaatagtcgttttgcatggatgactcggaagtctgaagaaacaattaccccatggaattttgaagaagttgtcgataaaggtgcttcagctcaatcatttattgaacgcatgacaaactttgataaaaatcttccaaatgaaaaagtactaccaaaacatagtttgctttatgagtattttacggtttataacgaattgacaaaggtcaaatatgttactgaaggaatgcgaaaaccagcatttctttcaggtgaacagaagaaagccattgttgatttactcttcaaaacaaatcgaaaagtaaccgttaagcaattaaaagaagattatttcaaaaaaatagaatgttttgatagtgttgaaatttcaggagttgaagatagatttaatgcttcattaggtacctaccatgatttgctaaaaattattaaagataaagattttttggataatgaagaaaatgaagatatcttagaggatattgttttaacattgaccttatttgaagatagggagatgattgaggaaagacttaaaacatatgctcacctctttgatgataaggtgatgaaacagcttaaacgtcgccgttatactggttggggacgtttgtctcgaaaattgattaatggtattagggataagcaatctggcaaaacaatattagattttttgaaatcagatggttttgccaatcgcaattttatgcagctgatccatgatgatagtttgacatttaaagaagacattcaaaaagcacaagtgtctggacaaggcgatagtttacatgaacatattgcaaatttagctggtagccctgctattaaaaaaggtattttacagactgtaaaagttgttgatgaattggtcaaagtaatggggcggcataagccagaaaatatcgttattgaaatggcacgtgaaaatcagacaactcaaaagggccagaaaaattcgcgagagcgtatgaaacgaatcgaagaaggtatcaaagaattaggaagtcagattcttaaagagcatcctgttgaaaatactcaattgcaaaatgaaaagctctatctctattatctccaaaatggaagagacatgtatgtggaccaagaattagatattaatcgtttaagtgattatgatgtcgatcacattgttccacaaagtttccttaaagacgattcaatagacaataaggtcttaacgcgttctgataaaaatcgtggtaaatcggataacgttccaagtgaagaagtagtcaaaaagatgaaaaactattggagacaacttctaaacgccaagttaatcactcaacgtaagtttgataatttaacgaaagctgaacgtggaggtttgagtgaacttgataaagctggttttatcaaacgccaattggttgaaactcgccaaatcactaagcatgtggcacaaattttggatagtcgcatgaatactaaatacgatgaaaatgataaacttattcgagaggttaaagtgattaccttaaaatctaaattagtttctgacttccgaaaagatttccaattctataaagtacgtgagattaacaattaccatcatgcccatgatgcgtatctaaatgccgtcgttggaactgctttgattaagaaatatccaaaacttgaatcggagtttgtctatggtgattataaagtttatgatgttcgtaaaatgattgctaagtctgagcaagaaataggcaaagcaaccgcaaaatatttcttttactctaatatcatgaacttcttcaaaacagaaattacacttgcaaatggagagattcgcaaacgccctctaatcgaaactaatggggaaactggagaaattgtctgggataaagggcgagattttgccacagtgcgcaaagtattgtccatgccccaagtcaatattgtcaagaaaacagaagtacagacaggcggattctccaaggagtcaattttaccaaaaagaaattcggacaagcttattgctcgtaaaaaagactgggatccaaaaaaatatggtggttttgatagtccaacggtagcttattcagtcctagtggttgctaaggtggaaaaagggaaatcgaagaagttaaaatccgttaaagagttactagggatcacaattatggaaagaagttcctttgaaaaaaatccgattgactttttagaagctaaaggatataaggaagttaaaaaagacttaatcattaaactacctaaatatagtctttttgagttagaaaacggtcgtaaacggatgctggctagtgccggagaattacaaaaaggaaatgagctggctctgccaagcaaatatgtgaattttttatatttagctagtcattatgaaaagttgaagggtagtccagaagataacgaacaaaaacaattgtttgtggagcagcataagcattatttagatgagattattgagcaaatcagtgaattttctaagcgtgttattttagcagatgccaatttagataaagttcttagtgcatataacaaacatagagacaaaccaatacgtgaacaagcagaaaatattattcatttatttacgttgacgaatcttggagctcccgctgcttttaaatattttgatacaacaattgatcgtaaacgatatacgtctacaaaagaagttttagatgccactcttatccatcaatccatcactggtctttatgaaacacgcattgatttgagtcagctaggaggtgactaacgcatcctcacgataatatccgggtaggcgcaatcactttcgtctactccgttacaaagcgaggctgggtatttcccggcctttctgttatccgaaatccactgaaagcacagcggctggctgaggagataaataataaacgaggggctgtatgcacaaagcatcttctgttgagttaagaacgagtatcgagatggcacatagccttgctcaaattggaatcaggtttgtgccaataccagtagaaacagacgaagaatccatgggtatggacagttttccctttgatatgtaacggtgaacagttgttctacttttgtttgttagtcttgatgcttcactgatagatacaagagccaaatctagtaatattttatctgattaataagatgatcttcttgagatcgttttggtctgcgcgtaatctcttgctctgaaaacgaaaaaaccgccttgcagggcggtttttcgaaggttctctgagctaccaactctttgaaccgaggtaactggcttggaggagcgcagtcaccaaaacttgtcctttcagtttagccttaaccggcgcatgacttcaagactaactcctctaaatcaattaccagtggctgctgccagtggtgcttttgcatgtctttccgggttggactcaagacgatagttaccggataaggcgcagcggtcggactgaacggggggttcgtgcatacagtccagcttggagcgaactgcctacccggaactgagtgtcaggcgtggaatgagacaaacgcggccataacagcggaatgacaccggtaaaccgaaaggcaggaacaggagagcgcacgagggagccgccagggggaaacgcctggtatctttatagtcctgtcgggtttcgccaccactgatttgagcgtcagatttcgtgatgcttgtcaggggggcggagcctatggaaaaacggctttgccgcggccccgctgaatattccttttgtctccgaccatcaggcacctgagtcgctgtctttttcgtgacattcagttcgctgcgctcacggctctggcagtgaatgggggtaaatggcactacaggcgccttttatggattcatgcaaggaaactacccataatacaagaaaagatgtggtctttattcttcaactaaagcacccattagttcaacaaacgaaaattggataaagtgggatatttttaaaatatatatttatgttacctggcagagcctgtactttttacagtcggttttctaatgtcactaacctgccccgttagtcgccatttgcatcgatttattatgacaacttgacggctacatcattcactttttcttcacaaccggcacggaactcgctcgggctggccccggtgcattttttaaatacccgcgagaaatagagttgatcgtcaaaaccaacattgcgaccgacggtggcgataggcatccgggtggtgctcaaaagcagcttcgcctggctgatacgttggtcctcgcgccagcttaagacgctaatccctaactgctggcggaaaagatgtgacagacgcgacggcgacaagcaaacatgctgtgcgacgctggcgatatcaaaattgctgtctgccaggtgatcgctgatgtactgacaagcctcgcgtacccgattatccatcggtggatggagcgactcgttaatcgcttccatgcgccgcagtaacaattgctcaagcagatttatcgccagcagctccgaatagcgcccttccccttgcccggcgttaatgatttgcccaaacaggtcgctgaaatgcggctggtgcgcttcatccgggcgaaagaaccccgtattggcaaatattgacggccagttaagccattcatgccagtaggcgcgcggacgaaagtaaacccactggtgataccattcgcgagcctccggatgacgaccgtagtgatgaatctctcctggcgggaacagcaaaatatcacccggtcggcaaacaaattctcgtccctgatttttcaccaccccctgaccgcgaatggtgagattgagaatataacctttcattcccagcggtcggtcgataaaaaaatcgagataaccgttggcctcaatcggcgttaaacccgccaccagatgggcattaaacgagtatcccggcagcaggggatcattttgcgcttcagccatacttttcatactcccgccattcagagaagaaaccaattgtccatattgcatcagacattgccgtcactgcgtcttttactggctcttctcgctaaccaaaccggtaaccccgcttattaaaagcattctgtaacaaagcgggaccagtaatagaaagtgagggagccacggttgatgagagctttgttgtaggtggaccagttggtgattttgaacttttgctttgccacggaacggtctgcgttgtcgggaagatgcgtgatctgatccttcaactcagcaaaagttcgatttattcaacaaagccacgttgtgtctcaaaatctctgatgttacattgcacaagataaaaatatatcatcatgaacaataaaactgtctgcttacataaacagtaatacaaggggtgttatgagccatattcaacgggaaacgtcttgctcgaggccgcgattaaattccaacatggatgctgatttatatgggtataaatgggctcgcgataatgtcgggcaatcaggtgcgacaatctatcgattgtatgggaagcccgatgcgccagagttgtttctgaaacatggcaaaggtagcgttgccaatgatgttacagatgagatggtcagactaaactggctgacggaatttatgcctcttccgaccatcaagcattttatccgtactcctgatgatgcatggttactcaccactgcgatccccgggaaaacagcattccaggtattagaagaatatcctgattcaggtgaaaatattgttgatgcgctggcagtgttcctgcgccggttgcattcgattcctgtttgtaattgtccttttaacagcgatcgcgtatttcgtctcgctcaggcgcaatcacgaatgaataacggtttggttgatgcgagtgattttgatgacgagcgtaatggctggcctgttgaacaagtctggaaagaaatgcataagcttttgccattctcaccggattcagtcgtcactcatggtgatttctcacttgataaccttatttttgacgaggggaaattaataggttgtattgatgttggacgagtcggaatcgcagaccgataccaggatcttgccatcctatggaactgcctcggtgagttttctccttcattacagaaacggctttttcaaaaatatggtattgataatcctgatatgaataaattgcagtttcatttgatgctcgatgagtttttctaatcagaattggttaattggttgtaaca